European Patent Application EP 4 191 335 A1, published June 7, 2023. Title: POLYPEPTIDE, PHOTORESIST COMPOSITION INCLUDING THE SAME, AND METHOD OF FORMING PATTERN USING THE SAME. Applicant: Samsung Electronics Co., Ltd. The sequence listing filed with the application follows.

SEQUENCE LISTING (14 sequences)

SEQ ID NO: 1 - protein, 6 aa, Artificial Sequence
  Artificial polypeptide
  FirstRepeatUnit1 (1)..(6)
GAGAGS

SEQ ID NO: 2 - protein, 4 aa, Artificial Sequence
  Artificial polypeptide
  FirstRepeatUnit2 (1)..(4)
GAAS

SEQ ID NO: 3 - protein, 4 aa, Artificial Sequence
  Artificial polypeptide
  SecondRepeatUnit1 (1)..(4)
GASY

SEQ ID NO: 4 - protein, 6 aa, Artificial Sequence
  Artificial polypeptide
  SecondRepeatUnit2 (1)..(6)
GAGASY

SEQ ID NO: 5 - protein, 8 aa, Artificial Sequence
  Artificial polypeptide
  SecondRepeatUnit3 (1)..(8)
GAGVGASY

SEQ ID NO: 6 - protein, 8 aa, Artificial Sequence
  Artificial polypeptide
  SecondRepeatUnit4 (1)..(8)
GAGAGASY

SEQ ID NO: 7 - protein, 10 aa, Artificial Sequence
  Artificial polypeptide
  RegionH1 (1)..(10)
GAGAGSGAAS

SEQ ID NO: 8 - protein, 4 aa, Artificial Sequence
  Artificial polypeptide
  RegionH2 (1)..(4)
GAAS

SEQ ID NO: 9 - protein, 42 aa, Artificial Sequence
  Artificial polypeptide
  SynthesisExample1 (1)..(42): HA1B4
GAGAGSGAASGAGAGSGAGAGYGAGVGAGYGAGYGAGAGAGY

SEQ ID NO: 10 - protein, 42 aa, Artificial Sequence
  Artificial polypeptide
  SynthesisExample2 (1)..(42): 14-A
GAGAGSGAASGAGAGSGAGAAYGAGVGAAYGAAYGAGAGAAY

SEQ ID NO: 11 - protein, 42 aa, Artificial Sequence
  Artificial polypeptide
  SynthesisExample3 (1)..(42): 14-P
GAGAGSGAASGAGAGSGAGAPYGAGVGAPYGAPYGAGAGAPY

SEQ ID NO: 12 - protein, 42 aa, Artificial Sequence
  Artificial polypeptide
  SynthesisExample4 (1)..(42): 14-S
GAGAGSGAASGAGAGSGAGASYGAGVGASYGASYGAGAGASY

SEQ ID NO: 13 - protein, 42 aa, Artificial Sequence
  Artificial polypeptide
  SynthesisExample5 (1)..(42): 14-D
GAGAGSGAASGAGAGSGAGADYGAGVGADYGADYGAGAGADY

SEQ ID NO: 14 - protein, 42 aa, Artificial Sequence
  Artificial polypeptide
  SynthesisExample6 (1)..(42): 14-K
GAGAGSGAASGAGAGSGAGAKYGAGVGAKYGAKYGAGAGAKY